European Patent Application EP 4 353 744 A1, published April 17, 2024. Title: ANTIBODY AGAINST RESPIRATORY SYNCYTIAL VIRUS AND USE THEREOF. Applicant: INSTITUTE OF MICROBIOLOGY, CHINESE ACADEMY OF SCIENCES. The sequence listing filed with the application follows.

SEQUENCE LISTING (32 sequences)

SEQ ID NO: 1 - protein, 564 aa, Artificial
  pre-fusion F protein
MELLILKANAITTILTAVTFCFASGQNITEEFYQSTCSAVSKGYLSALRTGWYTSVITIELSNIKENKCNGTDAKVKLIKQELDKYKNAVTELQLLMQSTPATNNRARRELPRFMNYTLNNTKKTNVTLSKKRKRRFLGFLLGVGSAIASGVAVCKVLHLEGEVNKIKSALLSTNKAVVSLSNGVSVLTFKVLDLKNYIDKQLLPILNKQSCSISNIETVIEFQQKNNRLLEITREFSVNAGVTTPVSTYMLTNSELLSLINDMPITNDQKKLMSNNVQIVRQQSYSIMCIIKEEVLAYVVQLPLYGVIDTPCWKLHTSPLCTTNTKEGSNICLTRTDRGWYCDNAGSVSFFPQAETCKVQSNRVFCDTMNSLTLPSEVNLCNVDIFNPKYDCKIMTSKTDVSSSVITSLGAIVSCYGKTKCTASNKNRGIIKTFSNGCDYVSNKGVDTVSVGNTLYYVNKQEGKSLYVKGEPIINFYDPLVFPSDEFDASISQVNEKINQSLAFIRKSDELLGSGYIPEAPRDGQAYVRKDGEWVLLSTFLLVPRGSHHHHHHGSWSHPQFGK

SEQ ID NO: 2 - protein, 118 aa, Artificial
  RV7 heavy chain variable region
QVQLQESGPGLVKPSETLSLTCTVSGGSISSYYLSWIRQPPGKGLEWIGYIYHTGSTNYNPSLKSRVTISVHSSKNQFSLKLTSVTAADTAVYYCARHMRIVTTIDYWGQGTLVTVSS

SEQ ID NO: 3 - protein, 107 aa, Artificial
  RV7 light chain variable region
DIVMTQSPSSLSASVGDRVTLTCRASQGISSYLAWYQQKPGKVPKLLIYAASTLQSGVPSRFSGSGSGTDFTLTISSLQPEDVATYYCQKYNSAPWTFGQGTKVEIK

SEQ ID NO: 4 - protein, 121 aa, Artificial
  RV8 heavy chain variable region
QVQLVQSGGGVVQPGRSLRLSCAASGFTFSSYAMHWVRQAPGKGLEWMAVISYDGSNTYYADSVKGRFTISRDNSKNTLYLQMNSLRAEDTAMFYCARDYCSRGTCYHDYWGQGTLVTVSS

SEQ ID NO: 5 - protein, 107 aa, Artificial
  RV8 light chain variable region
DIVLTQSPSSLSASVGDRVTITCRASQDIRNDLSWYQQKPGKAPKLLIYAASSLQSGVPSRFSGSGSGTDFTLTISSLQPEDFATYSCLQDYNYPQTFGQGTKVEIK

SEQ ID NO: 6 - protein, 118 aa, Artificial
  RV10 heavy chain variable region
QVQLVQSGAEVKKPGASVKVSCKASGYTFTTYDFHWVRQAPGQGLEWIGWLNPDNGNTKHSQKFQGRVTFTRDTSASTAFMELSSLRSEDTAVYYCTRAPWWWYFDYWGQGTLVTVSS

SEQ ID NO: 7 - protein, 115 aa, Artificial
  RV10 light chain variable region
NFMLTQPHSVSESPGKTVTISCTRSSGSIASNYVQWCQQRPGSSPTTVIYEDNQRPSGVPDRFSGSIDSSSNSASLTISGLRTEDEADYYCQSYDTSNAVFGGGTKLTVLGQPKA

SEQ ID NO: 8 - protein, 133 aa, Artificial
  RV11 heavy chain variable region
QVQLVQSGGGVVQPGRSLRLSCAASGFSFTNYGMHWVRQAPGKGLEWVAVISYDDGSDKYYADSVKGRFTISRDNSKNTLYLQMNSLRAEDTAVYYCVRDPTGDYGDFPEQDGYYYYYGMDVWGQGTTVTVSS

SEQ ID NO: 9 - protein, 115 aa, Artificial
  RV11 light chain variable region
QAVLTQPPSASGTPGQRVTISCSGSSLNIGSNYVYWYQQLPGTAPKFLIYKNNQRPSGVPDRFSGSKSGTSASLAISGLRSEDEADYYCAAWDDSLSGVVFGGGTKLTVLGQPKA

SEQ ID NO: 10 - protein, 330 aa, Artificial
  heavy chain constant region
ASTKGPSVFPLAPSSKSTSGGTAALGCLVKDYFPEPVTVSWNSGALTSGVHTFPAVLQSSGLYSLSSVVTVPSSSLGTQTYICNVNHKPSNTKVDKRVEPKSCDKTHTCPPCPAPELLGGPSVFLFPPKPKDTLMISRTPEVTCVVVDVSHEDPEVKFNWYVDGVEVHNAKTKPREEQYNSTYRVVSVLTVLHQDWLNGKEYKCKVSNKALPAPIEKTISKAKGQPREPQVYTLPPSRDELTKNQVSLTCLVKGFYPSDIAVEWESNGQPENNYKTTPPVLDSDGSFFLYSKLTVDKSRWQQGNVFSCSVMHEALHNHYTQKSLSLSPGK

SEQ ID NO: 11 - protein, 108 aa, Artificial
  light chain constant region CLκ
RTVAAPSVFIFPPSDEQLKSGTASVVCLLNNFYPREAKVQWKVDNALQSGNSQESVTEQDSKDSTYSLSSTLTLSKADYEKHKVYACEVTHQGLSSPVTKSFNRGECS

SEQ ID NO: 12 - protein, 101 aa, Artificial
  light chain constant region CLλ
APSVTLFPPSSEELQANKATLVCLISDFYPGAVTVAWKADSSPVKAGVETTTPSKQSNNKYAASSYLSLTPEQWKSHRSYSCQVTHEGSTVEKTVAPTECS

SEQ ID NO: 13 - protein, 20 aa, Artificial
  signal peptide
ETDTLLLWVLLLWVPGSTGD

SEQ ID NO: 14 - protein, 527 aa, Artificial
  post-fusion F protein
MELLILKANAITTILTAVTFCFASGQNITEEFYQSTCSAVSKGYLSALRTGWYTSVITIELSNIKENKCNGTDAKVKLIKQELDKYKNAVTELQLLMQSTPATNNRARRELPRFMNYTLNNAKKTNVTLSKKRKRRAIASGVAVSKVLHLEGEVNKIKSALLSTNKAVVSLSNGVSVLTSKVLDLKNYIDKQLLPIVNKQSCSISNIETVIEFQQKNNRLLEITREFSVNAGVTTPVSTYMLTNSELLSLINDMPITNDQKKLMSNNVQIVRQQSYSIMSIIKEEVLAYVVQLPLYGVIDTPCWKLHTSPLCTTNTKEGSNICLTRTDRGWYCDNAGSVSFFPQAETCKVQSNRVFCDTMNSLTLPSEVNLCNVDIFNPKYDCKIMTSKTDVSSSVITSLGAIVSCYGKTKCTASNKNRGIIKTFSNGCDYVSNKGVDTVSVGNTLYYVNKQEGKSLYVKGEPIINFYDPLVFPSDEFDASISQVNEKINQSLAFIRKSDELLLVPRGSHHHHHHHHGSWSHPQFGK

SEQ ID NO: 15 - protein, 6 aa, Artificial
  LCDR1
QDIRND

SEQ ID NO: 16 - protein, 3 aa, Artificial
  LCDR2
AAS

SEQ ID NO: 17 - protein, 11 aa, Artificial
  LCDR3
LQDYNYPQTFG

SEQ ID NO: 18 - protein, 8 aa, Artificial
  HCDR1
GFTFSSYA

SEQ ID NO: 19 - protein, 8 aa, Artificial
  HCDR2
ISYDGSNT

SEQ ID NO: 20 - protein, 14 aa, Artificial
  HCDR3
ARDYCSRGTCYHDY

SEQ ID NO: 21 - protein, 8 aa, Artificial
  LCDR1
SGSIASNY

SEQ ID NO: 22 - protein, 3 aa, Artificial
  LCDR2
EDN

SEQ ID NO: 23 - protein, 11 aa, Artificial
  LCDR3
QSYDTSNAVFG

SEQ ID NO: 24 - protein, 8 aa, Artificial
  HCDR1
GYTFTTYD

SEQ ID NO: 25 - protein, 8 aa, Artificial
  HCDR2
LNPDNGNT

SEQ ID NO: 26 - protein, 11 aa, Artificial
  HCDR3
TRAPWWWYFDY

SEQ ID NO: 27 - protein, 8 aa, Artificial
  LCDR1
SLNIGSNY

SEQ ID NO: 28 - protein, 3 aa, Artificial
  LCDR2
KNN

SEQ ID NO: 29 - protein, 13 aa, Artificial
  LCDR3
AAWDDSLSGVVFG

SEQ ID NO: 30 - protein, 8 aa, Artificial
  HCDR1
GFSFTNYG

SEQ ID NO: 31 - protein, 9 aa, Artificial
  HCDR2
ISYDDGSDK

SEQ ID NO: 32 - protein, 8 aa, Artificial
  HCDR3
VRDPTGDY